European Patent Application EP 4 183 405 A1, published May 24, 2023. Title: CRY1CA MUTANTS USEFUL FOR CONTROL OF INSECT PESTS. Applicant: Corteva Agriscience LLC. The sequence listing filed with the application follows.

SEQUENCE LISTING (40 sequences)

SEQ ID NO: 1 - DNA, 1878 bp, synthetic construct
  misc_feature 1..1878: note = synthesized coding region
  source 1..1878: mol_type = other DNA
atggataacaaccccaacattaacgagtgcatcccgtacaactgcctctcgaatccagaagaagtgctcttggatggcgagaggatttcgactggcaacagctccatcgacatttccctctccttggttcagttccttgtgtctaacttcgtccctggcggtggcttccttgttggccttatcgacttcgtctggggaattgtccagtgggatgcgtttctggtgcagatagagcagctgatcaacgagaggatcgctgagttcgcgagaaatgctgcaatcgccaaccttgaagggcttggcaacaacttcaacatctacgtggaggcgttcaaggagtgggaagaggaccctaagaatccagcgaccagaacgagggttatagatcggttccgcatcctcgatggccttttggagagggacatcccgagcttccgcatttcgggatttgaggttcctctgctctcagtctacgctcaagctgctaatctgcatctggccatcttgagggattcagtcatctttggcgaacgctggggtcttacgactatcaacgtgaacgagaactacaatcggttgattcggcacatagacgagtatgccgaccactgtgctaacacctacaataggggtctgaacaatctgccaaagtcaacgtatcaagactggataacctacaataggctcagacgggacctcactctcaccgtgctggacatagctgccttctttccgaactacgacaaccggagatatcctattcaacccgttggtcagctcactcgcgaggtctacaccgatcccctcatcaacttcaatccccagctgcaatcggtcgcacagctgcccaccttcaatgtgatggaaaactcagcgatccggaatccccatctgtttgacatacttaacaacctcactatcttcaccgattggttttcagttggacgcaacttctactggggagggcacagagtgatttcaagcctcattggaggagggaacattacatcgcctatctatggaagggaggccaaccaagagccaccaaggtctttcaccttcaacggtccggtgttcagaacacttagcaatcccacattgcgcttgctgcaacagccgtggccagcaccaccattcaatctgaggggagtggagggtgtggagttctcgacgcctacaaactcctttacgtacagaggcagagggacagtggactcactgacagaactcccacctgaggacaactctgttcctccgagggagggctactcgcaccggctttgccatgccaccttcgtccagaggtctggcacgccttttctgaccactggggttgtctttagctggactcaccgctcagcgacgctgaccaacacaatcgacccagagaggatcaatcagatccctctggtgaagggctttcgcgtttggggtggcacaagcgtgatcaccggacctggtttcactggtggggatatcctcagacgcaatacgtttggcgatttcgtgagccttcaagtcaacatcaattccccaatcacccagagatatcggctccgcttcagatacgcctcatccagagacgcaagggtcatcgtccttactggagcagccagcaccggagtcggaggccaagttagcgtcaacatgccgttgcagaaaacgatggaaatcggtgaaaacctcaccagcagaacctttcgctatacagatttcagcaaccctttctccttcagagccaatccggacataatcggcatatccgagcagcccttgttcggtgctgggtccatctcttctggcgagctgtacatcgacaagattgagatcattctcgcagatgcgactctggaggctgaatcggatcttgaaaggtga

SEQ ID NO: 2 - protein, 625 aa, synthetic construct
  REGION 1..625: note = translated from synthesized coding region
MDNNPNINECIPYNCLSNPEEVLLDGERISTGNSSIDISLSLVQFLVSNFVPGGGFLVGLIDFVWGIVQWDAFLVQIEQLINERIAEFARNAAIANLEGLGNNFNIYVEAFKEWEEDPKNPATRTRVIDRFRILDGLLERDIPSFRISGFEVPLLSVYAQAANLHLAILRDSVIFGERWGLTTINVNENYNRLIRHIDEYADHCANTYNRGLNNLPKSTYQDWITYNRLRRDLTLTVLDIAAFFPNYDNRRYPIQPVGQLTREVYTDPLINFNPQLQSVAQLPTFNVMENSAIRNPHLFDILNNLTIFTDWFSVGRNFYWGGHRVISSLIGGGNITSPIYGREANQEPPRSFTFNGPVFRTLSNPTLRLLQQPWPAPPFNLRGVEGVEFSTPTNSFTYRGRGTVDSLTELPPEDNSVPPREGYSHRLCHATFVQRSGTPFLTTGVVFSWTHRSATLTNTIDPERINQIPLVKGFRVWGGTSVITGPGFTGGDILRRNTFGDFVSLQVNINSPITQRYRLRFRYASSRDARVIVLTGAASTGVGGQVSVNMPLQKTMEIGENLTSRTFRYTDFSNPFSFRANPDIIGISEQPLFGAGSISSGELYIDKIEIILADATLEAESDLER

SEQ ID NO: 3 - DNA, 1878 bp, synthetic construct
  misc_feature 1..1878: note = synthesized coding region
  source 1..1878: mol_type = other DNA
atggataacaaccccaacattaacgagtgcatcccgtacaactgcctctcgaatccagaagaagtgctcttggatggcgagaggatttcgactggcaacagctccatcgacatttccctctccttggttcagttccttgtgtctaacttcgtccctggcgccggcttccttgttggccttatcgacttcgtctggggaattgtccagtgggatgcgtttctggtgcagatagagcagctgatcaacgagaggatcgctgagttcgcgagaaatgctgcaatcgccaaccttgaagggcttggcaacaacttcaacatctacgtggaggcgttcaaggagtgggaagaggaccctaagaatccagcgaccagaacgagggttatagatcggttccgcatcctcgatggccttttggagagggacatcccgagcttccgcatttcgggatttgaggttcctctgctctcagtctacgctcaagctgctaatctgcatctggccatcttgagggattcagtcatctttggcgaacgctggggtcttacgactatcaacgtgaacgagaactacaatcggttgattcggcacatagacgagtatgccgaccactgtgctaacacctacaataggggtctgaacaatctgccaaagtcaacgtatcaagactggataacctacaataggctcagacgggacctcactctcaccgtgctggacatagctgccttctttccgaactacgacaaccggagatatcctattcaacccgttggtcagctcactcgcgaggtctacaccgatcccctcatcaacttcaatccccagctgcaatcggtcgcacagctgcccaccttcaatgtgatggaaaactcagcgatccggaatccccatctgtttgacatacttaacaacctcactatcttcaccgattggttttcagttggacgcaacttctactggggagggcacagagtgatttcaagcctcattggaggagggaacattacatcgcctatctatggaagggaggccaaccaagagccaccaaggtctttcaccttcaacggtccggtgttcagaacacttagcaatcccacattgcgcttgctgcaacagccgtggccagcaccaccattcaatctgaggggagtggagggtgtggagttctcgacgcctacaaactcctttacgtacagaggcagagggacagtggactcactgacagaactcccacctgaggacaactctgttcctccgagggagggctactcgcaccggctttgccatgccaccttcgtccagaggtctggcacgccttttctgaccactggggttgtctttagctggactcaccgctcagcgacgctgaccaacacaatcgacccagagaggatcaatcagatccctctggtgaagggctttcgcgtttggggtggcacaagcgtgatcaccggacctggtttcactggtggggatatcctcagacgcaatacgtttggcgatttcgtgagccttcaagtcaacatcaattccccaatcacccagagatatcggctccgcttcagatacgcctcatccagagacgcaagggtcatcgtccttactggagcagccagcaccggagtcggaggccaagttagcgtcaacatgccgttgcagaaaacgatggaaatcggtgaaaacctcaccagcagaacctttcgctatacagatttcagcaaccctttctccttcagagccaatccggacataatcggcatatccgagcagcccttgttcggtgctgggtccatctcttctggcgagctgtacatcgacaagattgagatcattctcgcagatgcgactctggaggctgaatcggatcttgaaaggtga

SEQ ID NO: 4 - protein, 625 aa, synthetic construct
  REGION 1..625: note = translated from synthesized coding region
MDNNPNINECIPYNCLSNPEEVLLDGERISTGNSSIDISLSLVQFLVSNFVPGAGFLVGLIDFVWGIVQWDAFLVQIEQLINERIAEFARNAAIANLEGLGNNFNIYVEAFKEWEEDPKNPATRTRVIDRFRILDGLLERDIPSFRISGFEVPLLSVYAQAANLHLAILRDSVIFGERWGLTTINVNENYNRLIRHIDEYADHCANTYNRGLNNLPKSTYQDWITYNRLRRDLTLTVLDIAAFFPNYDNRRYPIQPVGQLTREVYTDPLINFNPQLQSVAQLPTFNVMENSAIRNPHLFDILNNLTIFTDWFSVGRNFYWGGHRVISSLIGGGNITSPIYGREANQEPPRSFTFNGPVFRTLSNPTLRLLQQPWPAPPFNLRGVEGVEFSTPTNSFTYRGRGTVDSLTELPPEDNSVPPREGYSHRLCHATFVQRSGTPFLTTGVVFSWTHRSATLTNTIDPERINQIPLVKGFRVWGGTSVITGPGFTGGDILRRNTFGDFVSLQVNINSPITQRYRLRFRYASSRDARVIVLTGAASTGVGGQVSVNMPLQKTMEIGENLTSRTFRYTDFSNPFSFRANPDIIGISEQPLFGAGSISSGELYIDKIEIILADATLEAESDLER

SEQ ID NO: 5 - DNA, 1878 bp, synthetic construct
  misc_feature 1..1878: note = synthesized coding region
  source 1..1878: mol_type = other DNA
atggataacaaccccaacattaacgagtgcatcccgtacaactgcctctcgaatccagaagaagtgctcttggatggcgagaggatttcgactggcaacagctccatcgacatttccctctccttggttcagttccttgtgtctaacttcgtccctggcggtggcttcgccgttggccttatcgacttcgtctggggaattgtccagtgggatgcgtttctggtgcagatagagcagctgatcaacgagaggatcgctgagttcgcgagaaatgctgcaatcgccaaccttgaagggcttggcaacaacttcaacatctacgtggaggcgttcaaggagtgggaagaggaccctaagaatccagcgaccagaacgagggttatagatcggttccgcatcctcgatggccttttggagagggacatcccgagcttccgcatttcgggatttgaggttcctctgctctcagtctacgctcaagctgctaatctgcatctggccatcttgagggattcagtcatctttggcgaacgctggggtcttacgactatcaacgtgaacgagaactacaatcggttgattcggcacatagacgagtatgccgaccactgtgctaacacctacaataggggtctgaacaatctgccaaagtcaacgtatcaagactggataacctacaataggctcagacgggacctcactctcaccgtgctggacatagctgccttctttccgaactacgacaaccggagatatcctattcaacccgttggtcagctcactcgcgaggtctacaccgatcccctcatcaacttcaatccccagctgcaatcggtcgcacagctgcccaccttcaatgtgatggaaaactcagcgatccggaatccccatctgtttgacatacttaacaacctcactatcttcaccgattggttttcagttggacgcaacttctactggggagggcacagagtgatttcaagcctcattggaggagggaacattacatcgcctatctatggaagggaggccaaccaagagccaccaaggtctttcaccttcaacggtccggtgttcagaacacttagcaatcccacattgcgcttgctgcaacagccgtggccagcaccaccattcaatctgaggggagtggagggtgtggagttctcgacgcctacaaactcctttacgtacagaggcagagggacagtggactcactgacagaactcccacctgaggacaactctgttcctccgagggagggctactcgcaccggctttgccatgccaccttcgtccagaggtctggcacgccttttctgaccactggggttgtctttagctggactcaccgctcagcgacgctgaccaacacaatcgacccagagaggatcaatcagatccctctggtgaagggctttcgcgtttggggtggcacaagcgtgatcaccggacctggtttcactggtggggatatcctcagacgcaatacgtttggcgatttcgtgagccttcaagtcaacatcaattccccaatcacccagagatatcggctccgcttcagatacgcctcatccagagacgcaagggtcatcgtccttactggagcagccagcaccggagtcggaggccaagttagcgtcaacatgccgttgcagaaaacgatggaaatcggtgaaaacctcaccagcagaacctttcgctatacagatttcagcaaccctttctccttcagagccaatccggacataatcggcatatccgagcagcccttgttcggtgctgggtccatctcttctggcgagctgtacatcgacaagattgagatcattctcgcagatgcgactctggaggctgaatcggatcttgaaaggtga

SEQ ID NO: 6 - protein, 625 aa, synthetic construct
  REGION 1..625: note = translated from synthesized coding region
MDNNPNINECIPYNCLSNPEEVLLDGERISTGNSSIDISLSLVQFLVSNFVPGGGFAVGLIDFVWGIVQWDAFLVQIEQLINERIAEFARNAAIANLEGLGNNFNIYVEAFKEWEEDPKNPATRTRVIDRFRILDGLLERDIPSFRISGFEVPLLSVYAQAANLHLAILRDSVIFGERWGLTTINVNENYNRLIRHIDEYADHCANTYNRGLNNLPKSTYQDWITYNRLRRDLTLTVLDIAAFFPNYDNRRYPIQPVGQLTREVYTDPLINFNPQLQSVAQLPTFNVMENSAIRNPHLFDILNNLTIFTDWFSVGRNFYWGGHRVISSLIGGGNITSPIYGREANQEPPRSFTFNGPVFRTLSNPTLRLLQQPWPAPPFNLRGVEGVEFSTPTNSFTYRGRGTVDSLTELPPEDNSVPPREGYSHRLCHATFVQRSGTPFLTTGVVFSWTHRSATLTNTIDPERINQIPLVKGFRVWGGTSVITGPGFTGGDILRRNTFGDFVSLQVNINSPITQRYRLRFRYASSRDARVIVLTGAASTGVGGQVSVNMPLQKTMEIGENLTSRTFRYTDFSNPFSFRANPDIIGISEQPLFGAGSISSGELYIDKIEIILADATLEAESDLER

SEQ ID NO: 7 - DNA, 1878 bp, synthetic construct
  misc_feature 1..1878: note = synthesized coding region
  source 1..1878: mol_type = other DNA
atggataacaaccccaacattaacgagtgcatcccgtacaactgcctctcgaatccagaagaagtgctcttggatggcgagaggatttcgactggcaacagctccatcgacatttccctctccttggttcagttccttgtgtctaacttcgtccctggcggtggcttcatggttggccttatcgacttcgtctggggaattgtccagtgggatgcgtttctggtgcagatagagcagctgatcaacgagaggatcgctgagttcgcgagaaatgctgcaatcgccaaccttgaagggcttggcaacaacttcaacatctacgtggaggcgttcaaggagtgggaagaggaccctaagaatccagcgaccagaacgagggttatagatcggttccgcatcctcgatggccttttggagagggacatcccgagcttccgcatttcgggatttgaggttcctctgctctcagtctacgctcaagctgctaatctgcatctggccatcttgagggattcagtcatctttggcgaacgctggggtcttacgactatcaacgtgaacgagaactacaatcggttgattcggcacatagacgagtatgccgaccactgtgctaacacctacaataggggtctgaacaatctgccaaagtcaacgtatcaagactggataacctacaataggctcagacgggacctcactctcaccgtgctggacatagctgccttctttccgaactacgacaaccggagatatcctattcaacccgttggtcagctcactcgcgaggtctacaccgatcccctcatcaacttcaatccccagctgcaatcggtcgcacagctgcccaccttcaatgtgatggaaaactcagcgatccggaatccccatctgtttgacatacttaacaacctcactatcttcaccgattggttttcagttggacgcaacttctactggggagggcacagagtgatttcaagcctcattggaggagggaacattacatcgcctatctatggaagggaggccaaccaagagccaccaaggtctttcaccttcaacggtccggtgttcagaacacttagcaatcccacattgcgcttgctgcaacagccgtggccagcaccaccattcaatctgaggggagtggagggtgtggagttctcgacgcctacaaactcctttacgtacagaggcagagggacagtggactcactgacagaactcccacctgaggacaactctgttcctccgagggagggctactcgcaccggctttgccatgccaccttcgtccagaggtctggcacgccttttctgaccactggggttgtctttagctggactcaccgctcagcgacgctgaccaacacaatcgacccagagaggatcaatcagatccctctggtgaagggctttcgcgtttggggtggcacaagcgtgatcaccggacctggtttcactggtggggatatcctcagacgcaatacgtttggcgatttcgtgagccttcaagtcaacatcaattccccaatcacccagagatatcggctccgcttcagatacgcctcatccagagacgcaagggtcatcgtccttactggagcagccagcaccggagtcggaggccaagttagcgtcaacatgccgttgcagaaaacgatggaaatcggtgaaaacctcaccagcagaacctttcgctatacagatttcagcaaccctttctccttcagagccaatccggacataatcggcatatccgagcagcccttgttcggtgctgggtccatctcttctggcgagctgtacatcgacaagattgagatcattctcgcagatgcgactctggaggctgaatcggatcttgaaaggtga

SEQ ID NO: 8 - protein, 625 aa, synthetic construct
  REGION 1..625: note = translated from synthesized coding region
MDNNPNINECIPYNCLSNPEEVLLDGERISTGNSSIDISLSLVQFLVSNFVPGGGFMVGLIDFVWGIVQWDAFLVQIEQLINERIAEFARNAAIANLEGLGNNFNIYVEAFKEWEEDPKNPATRTRVIDRFRILDGLLERDIPSFRISGFEVPLLSVYAQAANLHLAILRDSVIFGERWGLTTINVNENYNRLIRHIDEYADHCANTYNRGLNNLPKSTYQDWITYNRLRRDLTLTVLDIAAFFPNYDNRRYPIQPVGQLTREVYTDPLINFNPQLQSVAQLPTFNVMENSAIRNPHLFDILNNLTIFTDWFSVGRNFYWGGHRVISSLIGGGNITSPIYGREANQEPPRSFTFNGPVFRTLSNPTLRLLQQPWPAPPFNLRGVEGVEFSTPTNSFTYRGRGTVDSLTELPPEDNSVPPREGYSHRLCHATFVQRSGTPFLTTGVVFSWTHRSATLTNTIDPERINQIPLVKGFRVWGGTSVITGPGFTGGDILRRNTFGDFVSLQVNINSPITQRYRLRFRYASSRDARVIVLTGAASTGVGGQVSVNMPLQKTMEIGENLTSRTFRYTDFSNPFSFRANPDIIGISEQPLFGAGSISSGELYIDKIEIILADATLEAESDLER

SEQ ID NO: 9 - DNA, 1887 bp, Bacillus thuringiensis
  source 1..1887: mol_type = unassigned DNA
atggataacaaccccaacattaacgagtgcatcccgtacaactgcctctcgaatccagaagaagtgctcttggatggcgagaggatttcgactggcaacagctccatcgacatttccctctccttggttcagttccttgtgtctaacttcgtccctggcggtggcttccttgttggccttatcgacttcgtctggggaattgtcggaccctcccagtgggatgcgtttctggtgcagatagagcagctgatcaacgagaggatcgctgagttcgcgagaaatgctgcaatcgccaaccttgaagggcttggcaacaacttcaacatctacgtggaggcgttcaaggagtgggaagaggaccctaagaatccagcgaccagaacgagggttatagatcggttccgcatcctcgatggccttttggagagggacatcccgagcttccgcatttcgggatttgaggttcctctgctctcagtctacgctcaagctgctaatctgcatctggccatcttgagggattcagtcatctttggcgaacgctggggtcttacgactatcaacgtgaacgagaactacaatcggttgattcggcacatagacgagtatgccgaccactgtgctaacacctacaataggggtctgaacaatctgccaaagtcaacgtatcaagactggataacctacaataggctcagacgggacctcactctcaccgtgctggacatagctgccttctttccgaactacgacaaccggagatatcctattcaacccgttggtcagctcactcgcgaggtctacaccgatcccctcatcaacttcaatccccagctgcaatcggtcgcacagctgcccaccttcaatgtgatggaaaactcagcgatccggaatccccatctgtttgacatacttaacaacctcactatcttcaccgattggttttcagttggacgcaacttctactggggagggcacagagtgatttcaagcctcattggaggagggaacattacatcgcctatctatggaagggaggccaaccaagagccaccaaggtctttcaccttcaacggtccggtgttcagaacacttagcaatcccacattgcgcttgctgcaacagccgtggccagcaccaccattcaatctgaggggagtggagggtgtggagttctcgacgcctacaaactcctttacgtacagaggcagagggacagtggactcactgacagaactcccacctgaggacaactctgttcctccgagggagggctactcgcaccggctttgccatgccaccttcgtccagaggtctggcacgccttttctgaccactggggttgtctttagctggactcaccgctcagcgacgctgaccaacacaatcgacccagagaggatcaatcagatccctctggtgaagggctttcgcgtttggggtggcacaagcgtgatcaccggacctggtttcactggtggggatatcctcagacgcaatacgtttggcgatttcgtgagccttcaagtcaacatcaattccccaatcacccagagatatcggctccgcttcagatacgcctcatccagagacgcaagggtcatcgtccttactggagcagccagcaccggagtcggaggccaagttagcgtcaacatgccgttgcagaaaacgatggaaatcggtgaaaacctcaccagcagaacctttcgctatacagatttcagcaaccctttctccttcagagccaatccggacataatcggcatatccgagcagcccttgttcggtgctgggtccatctcttctggcgagctgtacatcgacaagattgagatcattctcgcagatgcgactctggaggctgaatcggatcttgaaaggtga

SEQ ID NO: 10 - protein, 628 aa, Bacillus thuringiensis
MDNNPNINECIPYNCLSNPEEVLLDGERISTGNSSIDISLSLVQFLVSNFVPGGGFLVGLIDFVWGIVGPSQWDAFLVQIEQLINERIAEFARNAAIANLEGLGNNFNIYVEAFKEWEEDPKNPATRTRVIDRFRILDGLLERDIPSFRISGFEVPLLSVYAQAANLHLAILRDSVIFGERWGLTTINVNENYNRLIRHIDEYADHCANTYNRGLNNLPKSTYQDWITYNRLRRDLTLTVLDIAAFFPNYDNRRYPIQPVGQLTREVYTDPLINFNPQLQSVAQLPTFNVMENSAIRNPHLFDILNNLTIFTDWFSVGRNFYWGGHRVISSLIGGGNITSPIYGREANQEPPRSFTFNGPVFRTLSNPTLRLLQQPWPAPPFNLRGVEGVEFSTPTNSFTYRGRGTVDSLTELPPEDNSVPPREGYSHRLCHATFVQRSGTPFLTTGVVFSWTHRSATLTNTIDPERINQIPLVKGFRVWGGTSVITGPGFTGGDILRRNTFGDFVSLQVNINSPITQRYRLRFRYASSRDARVIVLTGAASTGVGGQVSVNMPLQKTMEIGENLTSRTFRYTDFSNPFSFRANPDIIGISEQPLFGAGSISSGELYIDKIEIILADATLEAESDLER

SEQ ID NO: 11 - DNA, 1887 bp, synthetic construct
  misc_feature 1..1887: note = synthesized coding region
  source 1..1887: mol_type = other DNA
atggataacaaccccaacattaacgagtgcatcccgtacaactgcctctcgaatccagaagaagtgctcttggatggcgagaggatttcgactggcaacagctccatcgacatttccctctccttggttcagttccttgtgtctaacttcgtccctggcgccggcttccttgttggccttatcgacttcgtctggggaattgtcggaccctcccagtgggatgcgtttctggtgcagatagagcagctgatcaacgagaggatcgctgagttcgcgagaaatgctgcaatcgccaaccttgaagggcttggcaacaacttcaacatctacgtggaggcgttcaaggagtgggaagaggaccctaagaatccagcgaccagaacgagggttatagatcggttccgcatcctcgatggccttttggagagggacatcccgagcttccgcatttcgggatttgaggttcctctgctctcagtctacgctcaagctgctaatctgcatctggccatcttgagggattcagtcatctttggcgaacgctggggtcttacgactatcaacgtgaacgagaactacaatcggttgattcggcacatagacgagtatgccgaccactgtgctaacacctacaataggggtctgaacaatctgccaaagtcaacgtatcaagactggataacctacaataggctcagacgggacctcactctcaccgtgctggacatagctgccttctttccgaactacgacaaccggagatatcctattcaacccgttggtcagctcactcgcgaggtctacaccgatcccctcatcaacttcaatccccagctgcaatcggtcgcacagctgcccaccttcaatgtgatggaaaactcagcgatccggaatccccatctgtttgacatacttaacaacctcactatcttcaccgattggttttcagttggacgcaacttctactggggagggcacagagtgatttcaagcctcattggaggagggaacattacatcgcctatctatggaagggaggccaaccaagagccaccaaggtctttcaccttcaacggtccggtgttcagaacacttagcaatcccacattgcgcttgctgcaacagccgtggccagcaccaccattcaatctgaggggagtggagggtgtggagttctcgacgcctacaaactcctttacgtacagaggcagagggacagtggactcactgacagaactcccacctgaggacaactctgttcctccgagggagggctactcgcaccggctttgccatgccaccttcgtccagaggtctggcacgccttttctgaccactggggttgtctttagctggactcaccgctcagcgacgctgaccaacacaatcgacccagagaggatcaatcagatccctctggtgaagggctttcgcgtttggggtggcacaagcgtgatcaccggacctggtttcactggtggggatatcctcagacgcaatacgtttggcgatttcgtgagccttcaagtcaacatcaattccccaatcacccagagatatcggctccgcttcagatacgcctcatccagagacgcaagggtcatcgtccttactggagcagccagcaccggagtcggaggccaagttagcgtcaacatgccgttgcagaaaacgatggaaatcggtgaaaacctcaccagcagaacctttcgctatacagatttcagcaaccctttctccttcagagccaatccggacataatcggcatatccgagcagcccttgttcggtgctgggtccatctcttctggcgagctgtacatcgacaagattgagatcattctcgcagatgcgactctggaggctgaatcggatcttgaaaggtga

SEQ ID NO: 12 - protein, 628 aa, synthetic construct
  REGION 1..628: note = translated from synthesized coding region
MDNNPNINECIPYNCLSNPEEVLLDGERISTGNSSIDISLSLVQFLVSNFVPGAGFLVGLIDFVWGIVGPSQWDAFLVQIEQLINERIAEFARNAAIANLEGLGNNFNIYVEAFKEWEEDPKNPATRTRVIDRFRILDGLLERDIPSFRISGFEVPLLSVYAQAANLHLAILRDSVIFGERWGLTTINVNENYNRLIRHIDEYADHCANTYNRGLNNLPKSTYQDWITYNRLRRDLTLTVLDIAAFFPNYDNRRYPIQPVGQLTREVYTDPLINFNPQLQSVAQLPTFNVMENSAIRNPHLFDILNNLTIFTDWFSVGRNFYWGGHRVISSLIGGGNITSPIYGREANQEPPRSFTFNGPVFRTLSNPTLRLLQQPWPAPPFNLRGVEGVEFSTPTNSFTYRGRGTVDSLTELPPEDNSVPPREGYSHRLCHATFVQRSGTPFLTTGVVFSWTHRSATLTNTIDPERINQIPLVKGFRVWGGTSVITGPGFTGGDILRRNTFGDFVSLQVNINSPITQRYRLRFRYASSRDARVIVLTGAASTGVGGQVSVNMPLQKTMEIGENLTSRTFRYTDFSNPFSFRANPDIIGISEQPLFGAGSISSGELYIDKIEIILADATLEAESDLER

SEQ ID NO: 13 - DNA, 1887 bp, synthetic construct
  misc_feature 1..1887: note = synthesized coding region
  source 1..1887: mol_type = other DNA
atggataacaaccccaacattaacgagtgcatcccgtacaactgcctctcgaatccagaagaagtgctcttggatggcgagaggatttcgactggcaacagctccatcgacatttccctctccttggttcagttccttgtgtctaacttcgtccctggcggtggcttcatggttggccttatcgacttcgtctggggaattgtcggaccctcccagtgggatgcgtttctggtgcagatagagcagctgatcaacgagaggatcgctgagttcgcgagaaatgctgcaatcgccaaccttgaagggcttggcaacaacttcaacatctacgtggaggcgttcaaggagtgggaagaggaccctaagaatccagcgaccagaacgagggttatagatcggttccgcatcctcgatggccttttggagagggacatcccgagcttccgcatttcgggatttgaggttcctctgctctcagtctacgctcaagctgctaatctgcatctggccatcttgagggattcagtcatctttggcgaacgctggggtcttacgactatcaacgtgaacgagaactacaatcggttgattcggcacatagacgagtatgccgaccactgtgctaacacctacaataggggtctgaacaatctgccaaagtcaacgtatcaagactggataacctacaataggctcagacgggacctcactctcaccgtgctggacatagctgccttctttccgaactacgacaaccggagatatcctattcaacccgttggtcagctcactcgcgaggtctacaccgatcccctcatcaacttcaatccccagctgcaatcggtcgcacagctgcccaccttcaatgtgatggaaaactcagcgatccggaatccccatctgtttgacatacttaacaacctcactatcttcaccgattggttttcagttggacgcaacttctactggggagggcacagagtgatttcaagcctcattggaggagggaacattacatcgcctatctatggaagggaggccaaccaagagccaccaaggtctttcaccttcaacggtccggtgttcagaacacttagcaatcccacattgcgcttgctgcaacagccgtggccagcaccaccattcaatctgaggggagtggagggtgtggagttctcgacgcctacaaactcctttacgtacagaggcagagggacagtggactcactgacagaactcccacctgaggacaactctgttcctccgagggagggctactcgcaccggctttgccatgccaccttcgtccagaggtctggcacgccttttctgaccactggggttgtctttagctggactcaccgctcagcgacgctgaccaacacaatcgacccagagaggatcaatcagatccctctggtgaagggctttcgcgtttggggtggcacaagcgtgatcaccggacctggtttcactggtggggatatcctcagacgcaatacgtttggcgatttcgtgagccttcaagtcaacatcaattccccaatcacccagagatatcggctccgcttcagatacgcctcatccagagacgcaagggtcatcgtccttactggagcagccagcaccggagtcggaggccaagttagcgtcaacatgccgttgcagaaaacgatggaaatcggtgaaaacctcaccagcagaacctttcgctatacagatttcagcaaccctttctccttcagagccaatccggacataatcggcatatccgagcagcccttgttcggtgctgggtccatctcttctggcgagctgtacatcgacaagattgagatcattctcgcagatgcgactctggaggctgaatcggatcttgaaaggtga

SEQ ID NO: 14 - protein, 628 aa, synthetic construct
  REGION 1..628: note = translated from synthesized coding region
MDNNPNINECIPYNCLSNPEEVLLDGERISTGNSSIDISLSLVQFLVSNFVPGGGFMVGLIDFVWGIVGPSQWDAFLVQIEQLINERIAEFARNAAIANLEGLGNNFNIYVEAFKEWEEDPKNPATRTRVIDRFRILDGLLERDIPSFRISGFEVPLLSVYAQAANLHLAILRDSVIFGERWGLTTINVNENYNRLIRHIDEYADHCANTYNRGLNNLPKSTYQDWITYNRLRRDLTLTVLDIAAFFPNYDNRRYPIQPVGQLTREVYTDPLINFNPQLQSVAQLPTFNVMENSAIRNPHLFDILNNLTIFTDWFSVGRNFYWGGHRVISSLIGGGNITSPIYGREANQEPPRSFTFNGPVFRTLSNPTLRLLQQPWPAPPFNLRGVEGVEFSTPTNSFTYRGRGTVDSLTELPPEDNSVPPREGYSHRLCHATFVQRSGTPFLTTGVVFSWTHRSATLTNTIDPERINQIPLVKGFRVWGGTSVITGPGFTGGDILRRNTFGDFVSLQVNINSPITQRYRLRFRYASSRDARVIVLTGAASTGVGGQVSVNMPLQKTMEIGENLTSRTFRYTDFSNPFSFRANPDIIGISEQPLFGAGSISSGELYIDKIEIILADATLEAESDLER

SEQ ID NO: 15 - DNA, 1887 bp, synthetic construct
  misc_feature 1..1887: note = synthesized coding region
  source 1..1887: mol_type = other DNA
atggataacaaccccaacattaacgagtgcatcccgtacaactgcctctcgaatccagaagaagtgctcttggatggcgagaggatttcgactggcaacagctccatcgacatttccctctccttggttcagttccttgtgtctaacttcgtccctggcggtggcttcgccgttggccttatcgacttcgtctggggaattgtcggaccctcccagtgggatgcgtttctggtgcagatagagcagctgatcaacgagaggatcgctgagttcgcgagaaatgctgcaatcgccaaccttgaagggcttggcaacaacttcaacatctacgtggaggcgttcaaggagtgggaagaggaccctaagaatccagcgaccagaacgagggttatagatcggttccgcatcctcgatggccttttggagagggacatcccgagcttccgcatttcgggatttgaggttcctctgctctcagtctacgctcaagctgctaatctgcatctggccatcttgagggattcagtcatctttggcgaacgctggggtcttacgactatcaacgtgaacgagaactacaatcggttgattcggcacatagacgagtatgccgaccactgtgctaacacctacaataggggtctgaacaatctgccaaagtcaacgtatcaagactggataacctacaataggctcagacgggacctcactctcaccgtgctggacatagctgccttctttccgaactacgacaaccggagatatcctattcaacccgttggtcagctcactcgcgaggtctacaccgatcccctcatcaacttcaatccccagctgcaatcggtcgcacagctgcccaccttcaatgtgatggaaaactcagcgatccggaatccccatctgtttgacatacttaacaacctcactatcttcaccgattggttttcagttggacgcaacttctactggggagggcacagagtgatttcaagcctcattggaggagggaacattacatcgcctatctatggaagggaggccaaccaagagccaccaaggtctttcaccttcaacggtccggtgttcagaacacttagcaatcccacattgcgcttgctgcaacagccgtggccagcaccaccattcaatctgaggggagtggagggtgtggagttctcgacgcctacaaactcctttacgtacagaggcagagggacagtggactcactgacagaactcccacctgaggacaactctgttcctccgagggagggctactcgcaccggctttgccatgccaccttcgtccagaggtctggcacgccttttctgaccactggggttgtctttagctggactcaccgctcagcgacgctgaccaacacaatcgacccagagaggatcaatcagatccctctggtgaagggctttcgcgtttggggtggcacaagcgtgatcaccggacctggtttcactggtggggatatcctcagacgcaatacgtttggcgatttcgtgagccttcaagtcaacatcaattccccaatcacccagagatatcggctccgcttcagatacgcctcatccagagacgcaagggtcatcgtccttactggagcagccagcaccggagtcggaggccaagttagcgtcaacatgccgttgcagaaaacgatggaaatcggtgaaaacctcaccagcagaacctttcgctatacagatttcagcaaccctttctccttcagagccaatccggacataatcggcatatccgagcagcccttgttcggtgctgggtccatctcttctggcgagctgtacatcgacaagattgagatcattctcgcagatgcgactctggaggctgaatcggatcttgaaaggtga

SEQ ID NO: 16 - protein, 628 aa, synthetic construct
  REGION 1..628: note = translated from synthesized coding region
MDNNPNINECIPYNCLSNPEEVLLDGERISTGNSSIDISLSLVQFLVSNFVPGGGFAVGLIDFVWGIVGPSQWDAFLVQIEQLINERIAEFARNAAIANLEGLGNNFNIYVEAFKEWEEDPKNPATRTRVIDRFRILDGLLERDIPSFRISGFEVPLLSVYAQAANLHLAILRDSVIFGERWGLTTINVNENYNRLIRHIDEYADHCANTYNRGLNNLPKSTYQDWITYNRLRRDLTLTVLDIAAFFPNYDNRRYPIQPVGQLTREVYTDPLINFNPQLQSVAQLPTFNVMENSAIRNPHLFDILNNLTIFTDWFSVGRNFYWGGHRVISSLIGGGNITSPIYGREANQEPPRSFTFNGPVFRTLSNPTLRLLQQPWPAPPFNLRGVEGVEFSTPTNSFTYRGRGTVDSLTELPPEDNSVPPREGYSHRLCHATFVQRSGTPFLTTGVVFSWTHRSATLTNTIDPERINQIPLVKGFRVWGGTSVITGPGFTGGDILRRNTFGDFVSLQVNINSPITQRYRLRFRYASSRDARVIVLTGAASTGVGGQVSVNMPLQKTMEIGENLTSRTFRYTDFSNPFSFRANPDIIGISEQPLFGAGSISSGELYIDKIEIILADATLEAESDLER

SEQ ID NO: 17 - DNA, 1887 bp, synthetic construct
  misc_feature 1..1887: note = synthesized coding region
  source 1..1887: mol_type = other DNA
atggataacaaccccaacattaacgagtgcatcccgtacaactgcctctcgaatccagaagaagtgctcttggatggcgagaggatttcgactggcaacagctccatcgacatttccctctccttggttcagttccttgtgtctaacttcgtccctggcggtggcttccttgttggccttatcgacttcgtctggggaattttcggaccctcccagtgggatgcgtttctggtgcagatagagcagctgatcaacgagaggatcgctgagttcgcgagaaatgctgcaatcgccaaccttgaagggcttggcaacaacttcaacatctacgtggaggcgttcaaggagtgggaagaggaccctaagaatccagcgaccagaacgagggttatagatcggttccgcatcctcgatggccttttggagagggacatcccgagcttccgcatttcgggatttgaggttcctctgctctcagtctacgctcaagctgctaatctgcatctggccatcttgagggattcagtcatctttggcgaacgctggggtcttacgactatcaacgtgaacgagaactacaatcggttgattcggcacatagacgagtatgccgaccactgtgctaacacctacaataggggtctgaacaatctgccaaagtcaacgtatcaagactggataacctacaataggctcagacgggacctcactctcaccgtgctggacatagctgccttctttccgaactacgacaaccggagatatcctattcaacccgttggtcagctcactcgcgaggtctacaccgatcccctcatcaacttcaatccccagctgcaatcggtcgcacagctgcccaccttcaatgtgatggaaaactcagcgatccggaatccccatctgtttgacatacttaacaacctcactatcttcaccgattggttttcagttggacgcaacttctactggggagggcacagagtgatttcaagcctcattggaggagggaacattacatcgcctatctatggaagggaggccaaccaagagccaccaaggtctttcaccttcaacggtccggtgttcagaacacttagcaatcccacattgcgcttgctgcaacagccgtggccagcaccaccattcaatctgaggggagtggagggtgtggagttctcgacgcctacaaactcctttacgtacagaggcagagggacagtggactcactgacagaactcccacctgaggacaactctgttcctccgagggagggctactcgcaccggctttgccatgccaccttcgtccagaggtctggcacgccttttctgaccactggggttgtctttagctggactcaccgctcagcgacgctgaccaacacaatcgacccagagaggatcaatcagatccctctggtgaagggctttcgcgtttggggtggcacaagcgtgatcaccggacctggtttcactggtggggatatcctcagacgcaatacgtttggcgatttcgtgagccttcaagtcaacatcaattccccaatcacccagagatatcggctccgcttcagatacgcctcatccagagacgcaagggtcatcgtccttactggagcagccagcaccggagtcggaggccaagttagcgtcaacatgccgttgcagaaaacgatggaaatcggtgaaaacctcaccagcagaacctttcgctatacagatttcagcaaccctttctccttcagagccaatccggacataatcggcatatccgagcagcccttgttcggtgctgggtccatctcttctggcgagctgtacatcgacaagattgagatcattctcgcagatgcgactctggaggctgaatcggatcttgaaaggtga

SEQ ID NO: 18 - protein, 628 aa, synthetic construct
  REGION 1..628: note = translated from synthesized coding region
MDNNPNINECIPYNCLSNPEEVLLDGERISTGNSSIDISLSLVQFLVSNFVPGGGFLVGLIDFVWGIFGPSQWDAFLVQIEQLINERIAEFARNAAIANLEGLGNNFNIYVEAFKEWEEDPKNPATRTRVIDRFRILDGLLERDIPSFRISGFEVPLLSVYAQAANLHLAILRDSVIFGERWGLTTINVNENYNRLIRHIDEYADHCANTYNRGLNNLPKSTYQDWITYNRLRRDLTLTVLDIAAFFPNYDNRRYPIQPVGQLTREVYTDPLINFNPQLQSVAQLPTFNVMENSAIRNPHLFDILNNLTIFTDWFSVGRNFYWGGHRVISSLIGGGNITSPIYGREANQEPPRSFTFNGPVFRTLSNPTLRLLQQPWPAPPFNLRGVEGVEFSTPTNSFTYRGRGTVDSLTELPPEDNSVPPREGYSHRLCHATFVQRSGTPFLTTGVVFSWTHRSATLTNTIDPERINQIPLVKGFRVWGGTSVITGPGFTGGDILRRNTFGDFVSLQVNINSPITQRYRLRFRYASSRDARVIVLTGAASTGVGGQVSVNMPLQKTMEIGENLTSRTFRYTDFSNPFSFRANPDIIGISEQPLFGAGSISSGELYIDKIEIILADATLEAESDLER

SEQ ID NO: 19 - DNA, 1887 bp, synthetic construct
  misc_feature 1..1887: note = synthesized coding region
  source 1..1887: mol_type = other DNA
atggataacaaccccaacattaacgagtgcatcccgtacaactgcctctcgaatccagaagaagtgctcttggatggcgagaggatttcgactggcaacagctccatcgacatttccctctccttggttcagttccttgtgtctaacttcgtccctggcggtggcttccttgttggccttatcgacttcgtctggggaattatcggaccctcccagtgggatgcgtttctggtgcagatagagcagctgatcaacgagaggatcgctgagttcgcgagaaatgctgcaatcgccaaccttgaagggcttggcaacaacttcaacatctacgtggaggcgttcaaggagtgggaagaggaccctaagaatccagcgaccagaacgagggttatagatcggttccgcatcctcgatggccttttggagagggacatcccgagcttccgcatttcgggatttgaggttcctctgctctcagtctacgctcaagctgctaatctgcatctggccatcttgagggattcagtcatctttggcgaacgctggggtcttacgactatcaacgtgaacgagaactacaatcggttgattcggcacatagacgagtatgccgaccactgtgctaacacctacaataggggtctgaacaatctgccaaagtcaacgtatcaagactggataacctacaataggctcagacgggacctcactctcaccgtgctggacatagctgccttctttccgaactacgacaaccggagatatcctattcaacccgttggtcagctcactcgcgaggtctacaccgatcccctcatcaacttcaatccccagctgcaatcggtcgcacagctgcccaccttcaatgtgatggaaaactcagcgatccggaatccccatctgtttgacatacttaacaacctcactatcttcaccgattggttttcagttggacgcaacttctactggggagggcacagagtgatttcaagcctcattggaggagggaacattacatcgcctatctatggaagggaggccaaccaagagccaccaaggtctttcaccttcaacggtccggtgttcagaacacttagcaatcccacattgcgcttgctgcaacagccgtggccagcaccaccattcaatctgaggggagtggagggtgtggagttctcgacgcctacaaactcctttacgtacagaggcagagggacagtggactcactgacagaactcccacctgaggacaactctgttcctccgagggagggctactcgcaccggctttgccatgccaccttcgtccagaggtctggcacgccttttctgaccactggggttgtctttagctggactcaccgctcagcgacgctgaccaacacaatcgacccagagaggatcaatcagatccctctggtgaagggctttcgcgtttggggtggcacaagcgtgatcaccggacctggtttcactggtggggatatcctcagacgcaatacgtttggcgatttcgtgagccttcaagtcaacatcaattccccaatcacccagagatatcggctccgcttcagatacgcctcatccagagacgcaagggtcatcgtccttactggagcagccagcaccggagtcggaggccaagttagcgtcaacatgccgttgcagaaaacgatggaaatcggtgaaaacctcaccagcagaacctttcgctatacagatttcagcaaccctttctccttcagagccaatccggacataatcggcatatccgagcagcccttgttcggtgctgggtccatctcttctggcgagctgtacatcgacaagattgagatcattctcgcagatgcgactctggaggctgaatcggatcttgaaaggtga

SEQ ID NO: 20 - protein, 628 aa, synthetic construct
  REGION 1..628: note = translated from synthesized coding region
MDNNPNINECIPYNCLSNPEEVLLDGERISTGNSSIDISLSLVQFLVSNFVPGGGFLVGLIDFVWGIIGPSQWDAFLVQIEQLINERIAEFARNAAIANLEGLGNNFNIYVEAFKEWEEDPKNPATRTRVIDRFRILDGLLERDIPSFRISGFEVPLLSVYAQAANLHLAILRDSVIFGERWGLTTINVNENYNRLIRHIDEYADHCANTYNRGLNNLPKSTYQDWITYNRLRRDLTLTVLDIAAFFPNYDNRRYPIQPVGQLTREVYTDPLINFNPQLQSVAQLPTFNVMENSAIRNPHLFDILNNLTIFTDWFSVGRNFYWGGHRVISSLIGGGNITSPIYGREANQEPPRSFTFNGPVFRTLSNPTLRLLQQPWPAPPFNLRGVEGVEFSTPTNSFTYRGRGTVDSLTELPPEDNSVPPREGYSHRLCHATFVQRSGTPFLTTGVVFSWTHRSATLTNTIDPERINQIPLVKGFRVWGGTSVITGPGFTGGDILRRNTFGDFVSLQVNINSPITQRYRLRFRYASSRDARVIVLTGAASTGVGGQVSVNMPLQKTMEIGENLTSRTFRYTDFSNPFSFRANPDIIGISEQPLFGAGSISSGELYIDKIEIILADATLEAESDLER

SEQ ID NO: 21 - DNA, 1887 bp, synthetic construct
  misc_feature 1..1887: note = synthesized coding region
  source 1..1887: mol_type = other DNA
atggataacaaccccaacattaacgagtgcatcccgtacaactgcctctcgaatccagaagaagtgctcttggatggcgagaggatttcgactggcaacagctccatcgacatttccctctccttggttcagttccttgtgtctaacttcgtccctggcggtggcttccttgttggccttatcgacttcgtctggggaattgtcggaccctcccaggcggatgcgtttctggtgcagatagagcagctgatcaacgagaggatcgctgagttcgcgagaaatgctgcaatcgccaaccttgaagggcttggcaacaacttcaacatctacgtggaggcgttcaaggagtgggaagaggaccctaagaatccagcgaccagaacgagggttatagatcggttccgcatcctcgatggccttttggagagggacatcccgagcttccgcatttcgggatttgaggttcctctgctctcagtctacgctcaagctgctaatctgcatctggccatcttgagggattcagtcatctttggcgaacgctggggtcttacgactatcaacgtgaacgagaactacaatcggttgattcggcacatagacgagtatgccgaccactgtgctaacacctacaataggggtctgaacaatctgccaaagtcaacgtatcaagactggataacctacaataggctcagacgggacctcactctcaccgtgctggacatagctgccttctttccgaactacgacaaccggagatatcctattcaacccgttggtcagctcactcgcgaggtctacaccgatcccctcatcaacttcaatccccagctgcaatcggtcgcacagctgcccaccttcaatgtgatggaaaactcagcgatccggaatccccatctgtttgacatacttaacaacctcactatcttcaccgattggttttcagttggacgcaacttctactggggagggcacagagtgatttcaagcctcattggaggagggaacattacatcgcctatctatggaagggaggccaaccaagagccaccaaggtctttcaccttcaacggtccggtgttcagaacacttagcaatcccacattgcgcttgctgcaacagccgtggccagcaccaccattcaatctgaggggagtggagggtgtggagttctcgacgcctacaaactcctttacgtacagaggcagagggacagtggactcactgacagaactcccacctgaggacaactctgttcctccgagggagggctactcgcaccggctttgccatgccaccttcgtccagaggtctggcacgccttttctgaccactggggttgtctttagctggactcaccgctcagcgacgctgaccaacacaatcgacccagagaggatcaatcagatccctctggtgaagggctttcgcgtttggggtggcacaagcgtgatcaccggacctggtttcactggtggggatatcctcagacgcaatacgtttggcgatttcgtgagccttcaagtcaacatcaattccccaatcacccagagatatcggctccgcttcagatacgcctcatccagagacgcaagggtcatcgtccttactggagcagccagcaccggagtcggaggccaagttagcgtcaacatgccgttgcagaaaacgatggaaatcggtgaaaacctcaccagcagaacctttcgctatacagatttcagcaaccctttctccttcagagccaatccggacataatcggcatatccgagcagcccttgttcggtgctgggtccatctcttctggcgagctgtacatcgacaagattgagatcattctcgcagatgcgactctggaggctgaatcggatcttgaaaggtga

SEQ ID NO: 22 - protein, 628 aa, synthetic construct
  REGION 1..628: note = translated from synthesized coding region
MDNNPNINECIPYNCLSNPEEVLLDGERISTGNSSIDISLSLVQFLVSNFVPGGGFLVGLIDFVWGIVGPSQADAFLVQIEQLINERIAEFARNAAIANLEGLGNNFNIYVEAFKEWEEDPKNPATRTRVIDRFRILDGLLERDIPSFRISGFEVPLLSVYAQAANLHLAILRDSVIFGERWGLTTINVNENYNRLIRHIDEYADHCANTYNRGLNNLPKSTYQDWITYNRLRRDLTLTVLDIAAFFPNYDNRRYPIQPVGQLTREVYTDPLINFNPQLQSVAQLPTFNVMENSAIRNPHLFDILNNLTIFTDWFSVGRNFYWGGHRVISSLIGGGNITSPIYGREANQEPPRSFTFNGPVFRTLSNPTLRLLQQPWPAPPFNLRGVEGVEFSTPTNSFTYRGRGTVDSLTELPPEDNSVPPREGYSHRLCHATFVQRSGTPFLTTGVVFSWTHRSATLTNTIDPERINQIPLVKGFRVWGGTSVITGPGFTGGDILRRNTFGDFVSLQVNINSPITQRYRLRFRYASSRDARVIVLTGAASTGVGGQVSVNMPLQKTMEIGENLTSRTFRYTDFSNPFSFRANPDIIGISEQPLFGAGSISSGELYIDKIEIILADATLEAESDLER

SEQ ID NO: 23 - DNA, 1887 bp, synthetic construct
  misc_feature 1..1887: note = synthesized coding region
  source 1..1887: mol_type = other DNA
atggataacaaccccaacattaacgagtgcatcccgtacaactgcctctcgaatccagaagaagtgctcttggatggcgagaggatttcgactggcaacagctccatcgacatttccctctccttggttcagttccttgtgtctaacttcgtccctggcggtggcttccttgttggccttatcgacttcgtctggggaattgtcggaccctcccagtgggatgcgtttctggtgcagatagagcagctgatcaacgagaggatcgctgagttcgcgagaaatgctgcaatcgccaaccttgaagggcttggcaacaacttcaacatctacgtggaggcgttcaaggagtgggaagaggaccctaagaatccagcgaccagaacgagggttatagatcggttccgcatcctcgatggccttttggagagggacatcccgagcttccgcatttcgggatttgaggttcctctgctctcagtctacgctcaagctgctaatctgcatctggccatcttgagggattcagtcatctttggcgaacgctggggtcttacgactatcaacgtgaacgagaactacaatcggttgattcggcacatagacgagtatgccgaccactgtgctaacacctacaataggggtctgaacaatctgccaaagtcaacgtatcaagactggataacctacaataggctcagacgggacctcactctcaccgtgctggacatagctgccttctttccgaactacgacaaccggagatatcctattcaacccgttggtcagctcactcgcgaggtctacaccgatcccctcatcaacttcaatccccagctgcaatcggtcgcacagctgcccaccttcaatgtgatggaaaactcagcgatccggaatccccatctgtttgacatacttaacaacctcactatcttcaccgattggttttcagttggacgcaacttctactggggagggcacagagtgatttcaagcctcattggaggagggaacattacatcgcctatctatggaagggaggccaaccaagagccaccaaggtctttcaccttcaacggtccggtgttcagaacacttagcaatcccacattgcgcttgctgcaacagccgtggccagcaccaccattcaatctgaggggagtggagggtgtggagttctcgacgcctacaaactcctttacgtacagaggcagagggacagtggactcactgacagaactcccacctgaggacaactctgttcctccgagggagggctactcgcaccggctttgccatgccaccttcgtccagaggtctggcacgccttttctgaccactggggttgtctttagctggactcaccgctcagcgacgctgaccaacacaatcgacccagagaggatcaatcagatccctctggtgaagggctttcgcgtttggggtggcacaagcgtgatcaccggacctggtttcactggtggggatatcctcagacgcaatacgtttggcgatttcgtgagccttcaagtcaacatcaattccccaatcacccagagatatcggctccgcttcagatacgcctcatccagagacgcaagggtcatcgtccttactggagcagccagcaccggagtcggaggccaagttagcgtcaacatgccgttgcagaaaacgatggaaatcggtgaaaacctcaccagcagaacctttcgctatacagatttcagcaaccctttctccttcagagccaatccggacataatcggcatatccgagcagcccttgatgggtgctgggtccatctcttctggcgagctgtacatcgacaagattgagatcattctcgcagatgcgactctggaggctgaatcggatcttgaaaggtga

SEQ ID NO: 24 - protein, 628 aa, synthetic construct
  REGION 1..628: note = translated from synthesized coding region
MDNNPNINECIPYNCLSNPEEVLLDGERISTGNSSIDISLSLVQFLVSNFVPGGGFLVGLIDFVWGIVGPSQWDAFLVQIEQLINERIAEFARNAAIANLEGLGNNFNIYVEAFKEWEEDPKNPATRTRVIDRFRILDGLLERDIPSFRISGFEVPLLSVYAQAANLHLAILRDSVIFGERWGLTTINVNENYNRLIRHIDEYADHCANTYNRGLNNLPKSTYQDWITYNRLRRDLTLTVLDIAAFFPNYDNRRYPIQPVGQLTREVYTDPLINFNPQLQSVAQLPTFNVMENSAIRNPHLFDILNNLTIFTDWFSVGRNFYWGGHRVISSLIGGGNITSPIYGREANQEPPRSFTFNGPVFRTLSNPTLRLLQQPWPAPPFNLRGVEGVEFSTPTNSFTYRGRGTVDSLTELPPEDNSVPPREGYSHRLCHATFVQRSGTPFLTTGVVFSWTHRSATLTNTIDPERINQIPLVKGFRVWGGTSVITGPGFTGGDILRRNTFGDFVSLQVNINSPITQRYRLRFRYASSRDARVIVLTGAASTGVGGQVSVNMPLQKTMEIGENLTSRTFRYTDFSNPFSFRANPDIIGISEQPLMGAGSISSGELYIDKIEIILADATLEAESDLER

SEQ ID NO: 25 - DNA, 1887 bp, synthetic construct
  misc_feature 1..1887: note = synthesized coding region
  source 1..1887: mol_type = other DNA
atggataacaaccccaacattaacgagtgcatcccgtacaactgcctctcgaatccagaagaagtgctcttggatggcgagaggatttcgactggcaacagctccatcgacatttccctctccttggttcagttccttgtgtctaacttcgtccctggcggtggcttccttgttggccttatcgacttcgtctggggaattgtcggaccctcccagtgggatgcgtttctggtgcagatagagcagctgatcaacgagaggatcgctgagttcgcgagaaatgctgcaatcgccaaccttgaagggcttggcaacaacttcaacatctacgtggaggcgttcaaggagtgggaagaggaccctaagaatccagcgaccagaacgagggttatagatcggttccgcatcctcgatggccttttggagagggacatcccgagcttccgcatttcgggatttgaggttcctctgctctcagtctacgctcaagctgctaatctgcatctggccatcttgagggattcagtcatctttggcgaacgctggggtcttacgactatcaacgtgaacgagaactacaatcggttgattcggcacatagacgagtatgccgaccactgtgctaacacctacaataggggtctgaacaatctgccaaagtcaacgtatcaagactggataacctacaataggctcagacgggacctcactctcaccgtgctggacatagctgccttctttccgaactacgacaaccggagatatcctattcaacccgttggtcagctcactcgcgaggtctacaccgatcccctcatcaacttcaatccccagctgcaatcggtcgcacagctgcccaccttcaatgtgatggaaaactcagcgatccggaatccccatctgtttgacatacttaacaacctcactatcttcaccgattggttttcagttggacgcaacttctactggggagggcacagagtgatttcaagcctcattggaggagggaacattacatcgcctatctatggaagggaggccaaccaagagccaccaaggtctttcaccttcaacggtccggtgttcagaacacttagcaatcccacattgcgcttgctgcaacagccgtggccagcaccaccattcaatctgaggggagtggagggtgtggagttctcgacgcctacaaactcctttacgtacagaggcagagggacagtggactcactgacagaactcccacctgaggacaactctgttcctccgagggagggctactcgcaccggctttgccatgccaccttcgtccagaggtctggcacgccttttctgaccactggggttgtctttagctggactcaccgctcagcgacgctgaccaacacaatcgacccagagaggatcaatcagatccctctggtgaagggctttcgcgtttggggtggcacaagcgtgatcaccggacctggtttcactggtggggatatcctcagacgcaatacgtttggcgatttcgtgagccttcaagtcaacatcaattccccaatcacccagagatatcggctccgcttcagatacgcctcatccagagacgcaagggtcatcgtccttactggagcagccagcaccggagtcggaggccaagttagcgtcaacatgccgttgcagaaaacgatggaaatcggtgaaaacctcaccagcagaacctttcgctatacagatttcagcaaccctttctccttcagagccaatccggacataatcggcatatccgagcagcccttggccggtgctgggtccatctcttctggcgagctgtacatcgacaagattgagatcattctcgcagatgcgactctggaggctgaatcggatcttgaaaggtga

SEQ ID NO: 26 - protein, 628 aa, synthetic construct
  REGION 1..628: note = translated from synthesized coding region
MDNNPNINECIPYNCLSNPEEVLLDGERISTGNSSIDISLSLVQFLVSNFVPGGGFLVGLIDFVWGIVGPSQWDAFLVQIEQLINERIAEFARNAAIANLEGLGNNFNIYVEAFKEWEEDPKNPATRTRVIDRFRILDGLLERDIPSFRISGFEVPLLSVYAQAANLHLAILRDSVIFGERWGLTTINVNENYNRLIRHIDEYADHCANTYNRGLNNLPKSTYQDWITYNRLRRDLTLTVLDIAAFFPNYDNRRYPIQPVGQLTREVYTDPLINFNPQLQSVAQLPTFNVMENSAIRNPHLFDILNNLTIFTDWFSVGRNFYWGGHRVISSLIGGGNITSPIYGREANQEPPRSFTFNGPVFRTLSNPTLRLLQQPWPAPPFNLRGVEGVEFSTPTNSFTYRGRGTVDSLTELPPEDNSVPPREGYSHRLCHATFVQRSGTPFLTTGVVFSWTHRSATLTNTIDPERINQIPLVKGFRVWGGTSVITGPGFTGGDILRRNTFGDFVSLQVNINSPITQRYRLRFRYASSRDARVIVLTGAASTGVGGQVSVNMPLQKTMEIGENLTSRTFRYTDFSNPFSFRANPDIIGISEQPLAGAGSISSGELYIDKIEIILADATLEAESDLER

SEQ ID NO: 27 - DNA, 1887 bp, synthetic construct
  misc_feature 1..1887: note = synthesized coding region
  source 1..1887: mol_type = other DNA
atggataacaaccccaacattaacgagtgcatcccgtacaactgcctctcgaatccagaagaagtgctcttggatggcgagaggatttcgactggcaacagctccatcgacatttccctctccttggttcagttccttgtgtctaacttcgtccctggcgccggcttccttgttggccttatcgacttcgtctggggaattgtcggaccctcccagatggatgcgtttctggtgcagatagagcagctgatcaacgagaggatcgctgagttcgcgagaaatgctgcaatcgccaaccttgaagggcttggcaacaacttcaacatctacgtggaggcgttcaaggagtgggaagaggaccctaagaatccagcgaccagaacgagggttatagatcggttccgcatcctcgatggccttttggagagggacatcccgagcttccgcatttcgggatttgaggttcctctgctctcagtctacgctcaagctgctaatctgcatctggccatcttgagggattcagtcatctttggcgaacgctggggtcttacgactatcaacgtgaacgagaactacaatcggttgattcggcacatagacgagtatgccgaccactgtgctaacacctacaataggggtctgaacaatctgccaaagtcaacgtatcaagactggataacctacaataggctcagacgggacctcactctcaccgtgctggacatagctgccttctttccgaactacgacaaccggagatatcctattcaacccgttggtcagctcactcgcgaggtctacaccgatcccctcatcaacttcaatccccagctgcaatcggtcgcacagctgcccaccttcaatgtgatggaaaactcagcgatccggaatccccatctgtttgacatacttaacaacctcactatcttcaccgattggttttcagttggacgcaacttctactggggagggcacagagtgatttcaagcctcattggaggagggaacattacatcgcctatctatggaagggaggccaaccaagagccaccaaggtctttcaccttcaacggtccggtgttcagaacacttagcaatcccacattgcgcttgctgcaacagccgtggccagcaccaccattcaatctgaggggagtggagggtgtggagttctcgacgcctacaaactcctttacgtacagaggcagagggacagtggactcactgacagaactcccacctgaggacaactctgttcctccgagggagggctactcgcaccggctttgccatgccaccttcgtccagaggtctggcacgccttttctgaccactggggttgtctttagctggactcaccgctcagcgacgctgaccaacacaatcgacccagagaggatcaatcagatccctctggtgaagggctttcgcgtttggggtggcacaagcgtgatcaccggacctggtttcactggtggggatatcctcagacgcaatacgtttggcgatttcgtgagccttcaagtcaacatcaattccccaatcacccagagatatcggctccgcttcagatacgcctcatccagagacgcaagggtcatcgtccttactggagcagccagcaccggagtcggaggccaagttagcgtcaacatgccgttgcagaaaacgatggaaatcggtgaaaacctcaccagcagaacctttcgctatacagatttcagcaaccctttctccttcagagccaatccggacataatcggcatatccgagcagcccttgttcggtgctgggtccatctcttctggcgagctgtacatcgacaagattgagatcattctcgcagatgcgactctggaggctgaatcggatcttgaaaggtga

SEQ ID NO: 28 - protein, 628 aa, synthetic construct
  REGION 1..628: note = translated from synthesized coding region
MDNNPNINECIPYNCLSNPEEVLLDGERISTGNSSIDISLSLVQFLVSNFVPGAGFLVGLIDFVWGIVGPSQMDAFLVQIEQLINERIAEFARNAAIANLEGLGNNFNIYVEAFKEWEEDPKNPATRTRVIDRFRILDGLLERDIPSFRISGFEVPLLSVYAQAANLHLAILRDSVIFGERWGLTTINVNENYNRLIRHIDEYADHCANTYNRGLNNLPKSTYQDWITYNRLRRDLTLTVLDIAAFFPNYDNRRYPIQPVGQLTREVYTDPLINFNPQLQSVAQLPTFNVMENSAIRNPHLFDILNNLTIFTDWFSVGRNFYWGGHRVISSLIGGGNITSPIYGREANQEPPRSFTFNGPVFRTLSNPTLRLLQQPWPAPPFNLRGVEGVEFSTPTNSFTYRGRGTVDSLTELPPEDNSVPPREGYSHRLCHATFVQRSGTPFLTTGVVFSWTHRSATLTNTIDPERINQIPLVKGFRVWGGTSVITGPGFTGGDILRRNTFGDFVSLQVNINSPITQRYRLRFRYASSRDARVIVLTGAASTGVGGQVSVNMPLQKTMEIGENLTSRTFRYTDFSNPFSFRANPDIIGISEQPLFGAGSISSGELYIDKIEIILADATLEAESDLER

SEQ ID NO: 29 - DNA, 1887 bp, synthetic construct
  misc_feature 1..1887: note = synthesized coding region
  source 1..1887: mol_type = other DNA
atggataacaaccccaacattaacgagtgcatcccctacaactgcctctcgaatccagaagaagtgctcttggatggcgagaggatttcgactggcaacagctccatagacatttccctctccttggttcagttccttgtgtctaacttcgtccctggcggtggcttccttgttggattaatcgacttcgtctggggaattgtcggaccctcccagtgggatgcgtttctggtgcagatagagcaattaattaatgaaaggatcgctgagttcgcgagaaatgctgcaatcgccaaccttgaagggcttggcaacaacttcaacatctacgtggaagcatttaaggagtgggaagaggaccctaagaatccagcgaccagaacgagggttatagatcggttccgcatcctcgatggccttttggagagggacatcccgagcttccgcatttcgggatttgaggttcctctgctctcagtctacgctcaagctgctaatctgcatctggccatcttgagggattcagtcatctttggcgaacgctggggtcttacgactatcaacgtgaatgaaaactacaatcggttgattcggcacatagacgagtatgccgaccactgtgctaacacctacaataggggattaaataatctgccaaagtcaacgtatcaagactggataacatataataggctcagacgggacctcactctcaccgtgctggacatagctgccttctttccgaactacgacaaccggagatatcctattcaacccgttggtcagctcactcgcgaggtctacaccgatccattaattaatttcaatccccagctgcaatcggtcgcacagctgcccaccttcaatgtgatggaaaactcagcgatccggaatccccatctctttgacatacttaataatctcactatcttcaccgattggttttcagttggacgcaacttctactggggagggcacagagtgatttcaagcctcattggaggagggaacattacatcgcctatctatggaagggaggccaaccaggagccaccaaggtctttcaccttcaacggtccggtgttcagaacacttagcaatcccacattgcgcttgctgcaacagccgtggccagcaccaccattcaatctgaggggagtggagggtgtggagttctcgacgcctacaaactcctttacgtacagaggcagagggacagtggactcactgacagaactcccacctgaggacaactctgttcctccgagggagggctactcgcaccggctttgccatgccaccttcgtccagaggtctggcacgccttttctgaccactggggttgtctttagctggactcaccgctcagcgacgctgaccaatacaatcgacccagagagaattaatcaaatccctctggtgaagggctttcgcgtttggggtggcacaagcgtgatcaccggacctggtttcactggtggggatatcctcagacgcaatacgtttggcgatttcgtgagccttcaagtcaacattaattccccaatcacccagagatatcggctccgcttcagatacgcctcatccagagacgcaagggtcatcgtccttactggagcagccagcaccggagtcggaggccaagttagcgtcaacatgccgttgcagaaaacgatggaaatcggtgaaaacctcaccagcagaacctttcgctatacagatttcagcaaccctttctccttcagagccaatccggatataatcggcatatccgagcagcccttgttcggtgctgggtccatctcttcaggcgagctgtacatcgataaaattgagatcattctcgcagatgcgactctcgaggctgaatcggatcttgaaaggtga

SEQ ID NO: 30 - protein, 628 aa, Bacillus thuringiensis; identical to SEQ ID NO: 10

SEQ ID NO: 31 - DNA, 1887 bp, synthetic construct
  misc_feature 1..1887: note = synthesized coding region
  source 1..1887: mol_type = other DNA
atggataacaacccgaacatcaacgagtgcatcccctacaactgcctgagcaaccccgaggaggtgctgctggacggcgagaggatctcaaccggcaacagcagcatcgacatcagcctgtccctggtgcagttcctggtgagcaacttcgtgccgggcggcggcttcctggtgggattaatcgacttcgtgtggggcatcgtcggcccgtcccagtgggacgccttcctggttcagatcgagcaattaattaatgaaaggatagcagagttcgcgaggaacgcggccatcgccaacctggagggcctgggcaacaacttcaacatctacgtggaagcatttaaggagtgggaggaggaccccaagaacccggccacgaggacgagggtgatcgaccgctttcgcatcctggacggcctgctggagagggacatcccgtccttcagaatcagcggcttcgaggtcccgctgctgtccgtgtacgcgcaagcggccaacctgcacctggcgatcctgagggactccgtgatattcggcgagaggtggggcctgaccaccatcaacgtgaatgaaaactacaaccggctgataaggcacatcgacgagtacgccgaccactgcgccaacacctacaataggggattaaataatctgcccaagagcacctaccaagactggatcacatataaccggctgaggagggacctgaccctgaccgtgctggacatcgccgcgttcttcccgaactacgacaataggcgctacccgatccagccggtgggccagctgacccgcgaggtgtacaccgacccattaattaatttcaacccgcagctccagtccgtggcccagctgccgaccttcaacgtgatggagaacagcgccatccggaacccgcacctgttcgacatcctgaataatctgaccatcttcaccgactggttctcagtgggccggaacttctactggggcggccatagggtgatctccagcctgatcggcggcggcaacatcacctccccgatctacgggagggaggcgaaccaggagccgccgaggtccttcaccttcaacggcccggtgtttaggaccctgtccaacccgaccctgaggctgctccagcagccgtggccggcgccgccgttcaacctgaggggcgtggagggcgtggagttcagcaccccgaccaacagcttcacctaccgggggaggggcaccgtggactcactgaccgagctgccgccggaggacaacagcgtgccgccgagggagggctacagccataggctgtgccacgccaccttcgtgcagaggagcggcaccccgttcttgacgaccggcgtggtgttctcctggacccaccggagcgcgaccctgaccaatacaatcgacccggagagaattaatcaaatcccgctggtgaagggcttccgggtgtggggcggcacctccgtgatcaccgggccgggctttaccggcggcgacatcctgaggaggaacacgttcggcgacttcgtgagcctccaagtgaacattaatagcccgatcacccagcgctaccggctgaggttccgctacgcgtcaagccgcgacgcgagggtgatcgtgctgaccggcgcggcctcaaccggcgtgggcggccaagtgtccgtgaacatgccgctgcaaaagacgatggagatcggcgagaacctgacctcaaggaccttccgctacaccgacttcagcaacccgttcagctttagggccaacccggatataatcggcatcagcgagcagccgctgttcggcgccggctccatctcaagcggcgagctgtacatcgataaaatcgagatcatcctggcggacgcgaccttggaggccgagtccgacctggagaggtga

SEQ ID NO: 32 - protein, 628 aa, Bacillus thuringiensis; identical to SEQ ID NO: 10

SEQ ID NO: 33 - DNA, 1887 bp, synthetic construct
  misc_feature 1..1887: note = synthesized coding region
  source 1..1887: mol_type = other DNA
atggacaacaatcccaatatcaatgagtgcatcccatacaactgcctttcaaatcccgaggaagtcttactggatggggaaaggattagcactggcaattccagcattgacatttccttgagtctcgttcaattccttgtgagcaactttgtgcctggcggagggttcttggttggtctcatagactttgtttggggaattgtaggaccatcacagtgggatgccttcttagtccagattgaacagcttatcaatgagagaatagctgagttcgcaagaaatgctgcaatcgctaacttggagggactcggcaacaacttcaacatctacgtggaggctttcaaagaatgggaagaagatcctaagaatccagctactaggactagagtcatcgataggtttaggattcttgatgggctgttggagcgtgacattccttcctttaggattagtggcttcgaggttcctctcctttctgtctatgctcaagcagccaatctccatctcgccattctccgtgattcagtaatcttcggagaaagatggggtttgacaacgatcaatgtgaatgagaactacaacagattgatcagacacattgatgagtatgctgatcattgtgctaacacatacaacagagggcttaacaacctcccgaaatcaacatatcaagattggataacctacaatagattgaggagggatctcacactgactgtactcgacattgctgctttctttcccaactacgataaccgtagatatcccattcaacccgtcggacaactcactcgtgaagtgtacacagatccccttatcaacttcaacccacagttacaaagtgttgcacagctgccaaccttcaatgtgatggaaaactctgccattaggaatccacatctgtttgacatacttaacaacttgactatctttacggattggtttagtgtggggaggaacttctattggggaggtcacagagtgattagctctcttatcggaggtgggaacattacttcaccaatctatggacgtgaagcaaatcaagaaccaccacgttcattcaccttcaatggacccgttttcagaacactgtccaatccgactctgagactgttgcagcaaccttggccagcacctcctttcaacttgaggggtgtagagggagtcgagttttccacacctactaacagtttcacctataggggtcgtggaactgttgattctcttactgaacttcctccagaggacaattctgttcctccgagggaaggctattcacaccgtttgtgtcatgcaacttttgttcagaggtctggcacacctttcttaacaactggcgtcgttttcagctggacacataggagtgcaaccctcacgaatactatcgatccagagagaatcaatcagattcctcttgttaagggctttagggtgtggggtgggacctcagtgataactggtcccggtttcaccggaggagacatacttagaaggaacacctttggggatttcgtttctcttcaagtaaacatcaattctcctatcacccagagatacagacttaggtttagatatgctagtagccgtgacgccagagtcatagtgttgactggtgctgcatcaactggtgttggtgggcaagtttcagtgaacatgccacttcaaaagacaatggagataggtgagaacttgacgtccagaaccttcagatacactgacttttctaatcctttctcttttcgtgctaatccagacatcataggaatcagtgaacaaccgttgtttggagctggttccatttctagtggagaattgtacattgacaagattgagatcatacttgccgatgccacgctcgaggctgaatctgatctcgaaaggtga

SEQ ID NO: 34 - protein, 628 aa, Bacillus thuringiensis; identical to SEQ ID NO: 10

SEQ ID NO: 35 - DNA, 3495 bp, synthetic construct
  misc_feature 1..3495: note = synthesized coding region
  source 1..3495: mol_type = other DNA
atggacaacaatcccaatatcaatgagtgcatcccatacaactgcctttcaaatcccgaggaagtcttactggatggggaaaggattagcactggcaattccagcattgacatttccttgagtctcgttcaattccttgtgagcaactttgtgcctggcggagggttcttggttggtctcatagactttgtttggggaattgtaggaccatcacagtgggatgccttcttagtccagattgaacagcttatcaatgagagaatagctgagttcgcaagaaatgctgcaatcgctaacttggagggactcggcaacaacttcaacatctacgtggaggctttcaaagaatgggaagaagatcctaagaatccagctactaggactagagtcatcgataggtttaggattcttgatgggctgttggagcgtgacattccttcctttaggattagtggcttcgaggttcctctcctttctgtctatgctcaagcagccaatctccatctcgccattctccgtgattcagtaatcttcggagaaagatggggtttgacaacgatcaatgtgaatgagaactacaacagattgatcagacacattgatgagtatgctgatcattgtgctaacacatacaacagagggcttaacaacctcccgaaatcaacatatcaagattggataacctacaatagattgaggagggatctcacactgactgtactcgacattgctgctttctttcccaactacgataaccgtagatatcccattcaacccgtcggacaactcactcgtgaagtgtacacagatccccttatcaacttcaacccacagttacaaagtgttgcacagctgccaaccttcaatgtgatggaaaactctgccattaggaatccacatctgtttgacatacttaacaacttgactatctttacggattggtttagtgtggggaggaacttctattggggaggtcacagagtgattagctctcttatcggaggtgggaacattacttcaccaatctatggacgtgaagcaaatcaagaaccaccacgttcattcaccttcaatggacccgttttcagaacactgtccaatccgactctgagactgttgcagcaaccttggccagcacctcctttcaacttgaggggtgtagagggagtcgagttttccacacctactaacagtttcacctataggggtcgtggaactgttgattctcttactgaacttcctccagaggacaattctgttcctccgagggaaggctattcacaccgtttgtgtcatgcaacttttgttcagaggtctggcacacctttcttaacaactggcgtcgttttcagctggacacataggagtgcaaccctcacgaatactatcgatccagagagaatcaatcagattcctcttgttaagggctttagggtgtggggtgggacctcagtgataactggtcccggtttcaccggaggagacatacttagaaggaacacctttggggatttcgtttctcttcaagtaaacatcaattctcctatcacccagagatacagacttaggtttagatatgctagtagccgtgacgccagagtcatagtgttgactggtgctgcatcaactggtgttggtgggcaagtttcagtgaacatgccacttcaaaagacaatggagataggtgagaacttgacgtccagaaccttcagatacactgacttttctaatcctttctcttttcgtgctaatccagacatcataggaatcagtgaacaaccgttgtttggagctggttccatttctagtggagaattgtacattgacaagattgagatcatacttgccgatgccacgctcgaggctgaatctgatctcgaaagggcacagaaagctgtaaacgcattgtttacaagttctaatcaaatcggactcaaaaccgatgttacggactatcacatagatagggtttctaatcttgtggaatgtctttcagatgagttttgtttagatgagaagaaagaactttcagaaaaggtcaagcacgccaaaagactgtccgatgaaaggaatctccttcaagacccaaactttcgtggaatcaataggcagctcgacagaggttggagagggagcacagatatcaccattcaaggaggagatgacgttttcaaagagaactatgtcaccttgttaggcacctttgatgagtgctatccaacttatctgtatcagaagattgatgaatccaagctgaaggcttacacaagatatcagctcagaggatacatcgaggactcccaagatttggagatatacttgattcgttacaatgcaaaacatgagaccgtgaatgttcctggtactggaagtctctggccactgtctgctccgtcacctattgggaaatgtgcccatcactcccaccatttctcattggacatagacgttggctgcacagatttgaatgaagatttgggtgtttgggtcatcttcaagatcaaaactcaagacggacacgctcgtttaggaaacttagagtttcttgaagagaagcccttggttggggaggcacttgccagagtaaagagagctgaaaagaagtggagagataagagggagaaacttgagtgggagactaacattgtgtacaaggaagccaaagaaagcgtggatgctcttttcgtgaactctcagtatgataggttacaagcagacaccaacatagcaatgatacatgcagctgacaaaagagtccattctattcgtgaggcttacttgccagaacttagtgtgattcccggtgtcaacgctgccattttcgaggaattggaaggaagaatctttacggctttcagcctctatgacgctaggaatgttatcaagaatggtgatttcaacaatggcctctcatgttggaatgtgaaaggtcatgttgatgtagaggagcaaaacaatcaccgtagcgtgctggttgtcccagaatgggaagccgaagtaagccaagaagttagagtttgccctggaagaggctacattctgcgtgtcaccgcttacaaagaaggatatggcgaagggtgcgtgactattcatgagattgagaacaatactgacgaacttaagttttcaaactgcgtcgaggaggaagtgtatcctaacaacacagtgacttgtaatgactatacagcaacgcaagaggaatacgaggggacatacaccagtcgtaatcgtggttatgatggtgcttatgaaagcaattcatccgttccagctgactatgccagtgcctacgaagagaaggcttacacggatggcagaagagataacccatgtgagtccaacagaggttatggtgattacactcctcttccagctggttacgtgactaaagagttagagtactttccggagactgataaggtttggattgaaatcggagagacagaagggacattcatagtagattcagttgagcttcttctcatggaagaatga

SEQ ID NO: 36 - protein, 1164 aa, synthetic construct
  REGION 1..1164: note = translated from synthesized coding region
MDNNPNINECIPYNCLSNPEEVLLDGERISTGNSSIDISLSLVQFLVSNFVPGGGFLVGLIDFVWGIVGPSQWDAFLVQIEQLINERIAEFARNAAIANLEGLGNNFNIYVEAFKEWEEDPKNPATRTRVIDRFRILDGLLERDIPSFRISGFEVPLLSVYAQAANLHLAILRDSVIFGERWGLTTINVNENYNRLIRHIDEYADHCANTYNRGLNNLPKSTYQDWITYNRLRRDLTLTVLDIAAFFPNYDNRRYPIQPVGQLTREVYTDPLINFNPQLQSVAQLPTFNVMENSAIRNPHLFDILNNLTIFTDWFSVGRNFYWGGHRVISSLIGGGNITSPIYGREANQEPPRSFTFNGPVFRTLSNPTLRLLQQPWPAPPFNLRGVEGVEFSTPTNSFTYRGRGTVDSLTELPPEDNSVPPREGYSHRLCHATFVQRSGTPFLTTGVVFSWTHRSATLTNTIDPERINQIPLVKGFRVWGGTSVITGPGFTGGDILRRNTFGDFVSLQVNINSPITQRYRLRFRYASSRDARVIVLTGAASTGVGGQVSVNMPLQKTMEIGENLTSRTFRYTDFSNPFSFRANPDIIGISEQPLFGAGSISSGELYIDKIEIILADATLEAESDLERAQKAVNALFTSSNQIGLKTDVTDYHIDRVSNLVECLSDEFCLDEKKELSEKVKHAKRLSDERNLLQDPNFRGINRQLDRGWRGSTDITIQGGDDVFKENYVTLLGTFDECYPTYLYQKIDESKLKAYTRYQLRGYIEDSQDLEIYLIRYNAKHETVNVPGTGSLWPLSAPSPIGKCAHHSHHFSLDIDVGCTDLNEDLGVWVIFKIKTQDGHARLGNLEFLEEKPLVGEALARVKRAEKKWRDKREKLEWETNIVYKEAKESVDALFVNSQYDRLQADTNIAMIHAADKRVHSIREAYLPELSVIPGVNAAIFEELEGRIFTAFSLYDARNVIKNGDFNNGLSCWNVKGHVDVEEQNNHRSVLVVPEWEAEVSQEVRVCPGRGYILRVTAYKEGYGEGCVTIHEIENNTDELKFSNCVEEEVYPNNTVTCNDYTATQEEYEGTYTSRNRGYDGAYESNSSVPADYASAYEEKAYTDGRRDNPCESNRGYGDYTPLPAGYVTKELEYFPETDKVWIEIGETEGTFIVDSVELLLMEE

SEQ ID NO: 37 - DNA, 3495 bp, synthetic construct
  misc_feature 1..3495: note = synthesized coding region
  source 1..3495: mol_type = other DNA
atggataacaatccgaacatcaatgaatgcatcccgtacaactgcctgagcaacccggaagaagtgctgttggatggagaacggatatcaactggtaattcatcaattgatatttctctgtcacttgttcagtttctggtatctaacttcgtcccaggcggaggattcctggttggattaatagattttgtatggggaatagttggcccttctcaatgggatgcatttctagtacaaattgaacaattaattaatgaaagaatagctgaatttgctaggaatgctgctattgctaatttagaaggattaggaaacaatttcaatatatatgtggaagcatttaaagaatgggaagaagatcctaagaatccagcaaccaggaccagagtaattgatcgctttcgtatacttgatgggctacttgaaagggacattccttcgtttcgaatttctggatttgaagtaccccttttatccgtttatgctcaagcggccaatctgcatctagctatattaagagattctgtaatttttggagaaagatggggattgacaacgataaatgtcaatgaaaactataatagactaattaggcatattgatgaatatgctgatcactgtgcaaatacgtataatcggggattaaataatttaccgaaatctacgtatcaagattggataacatataatcgattgcggagagacttaacattgactgtattagatatcgccgctttctttccaaactatgacaataggagatatccaattcagccagttggtcaactaacaagggaagtttatacggacccattaattaattttaatccacagttacagtctgtagctcaattacctacttttaacgttatggagaacagcgcaattagaaatcctcatttatttgatatattgaataatcttacaatctttacggattggtttagtgttggacgcaatttttattggggaggacatcgagtaatatctagccttataggaggtggtaacataacatctcctatatatggaagagaggcgaaccaggagcctccaagatcctttacttttaatggaccggtatttaggactttatcaaatcctactttacgattattacagcaaccttggccagcgccaccatttaatttacgtggtgttgaaggagtagaattttctacacctacaaatagctttacgtatcgaggaagaggtacggttgattctttaactgaattgccgcctgaggataatagtgtgccacctcgcgaaggatatagtcatcgtttatgtcatgcaacttttgttcaaagatctggaacaccttttttaacaactggtgtagtattttcttggacgcatcgtagtgcaactcttacaaatacaattgatccagagagaattaatcaaatacctttagtgaaaggatttagagtttgggggggcacctctgtcattacaggaccaggatttacaggaggggatatccttcgaagaaatacctttggtgattttgtatctctacaagtcaatattaattcaccaattacccaaagataccgtttaagatttcgttacgcttccagtagggatgcacgagttatagtattaacaggagcggcatccacaggagtgggaggccaagttagtgtaaatatgcctcttcagaaaactatggaaataggggagaacttaacatctagaacatttagatataccgattttagtaatcctttttcatttagagctaatccagatataattgggataagtgaacaacctctatttggtgcaggttctattagtagcggtgaactttatatagataaaattgaaattattctagcagatgcaacatttgaagcagaatctgatttagaaagagcacaaaaggcggtgaatgccctgtttacttcttccaatcaaatcgggttaaaaaccgatgtgacggactatcatatcgatcgagtatccaatttagttgagtgtttatctgatgaattttgtctggatgaaaaaaaagaattgtccgagaaagtcaaacatgcgaagcgacttagtgatgagcggaatttacttcaagatccaaactttagagggatcaatagacaactagaccgtggctggagaggaagtacggatattaccatccaaggaggcgatgacgtatccaaagagaattacgttacgctattgggtacctttgatgagtgctacttaacgtatttatatcaaaaaatagatgagtcgaaattaaaagcctatacccgttaccaattaagagggtatatcgaagatagtcaagacttagaaatctatttaattcgctacaatgccaaacacgaaacagtaaatgtgccaggtacgggttccttatggccgctttcagccccaagtccaatcggaaaatgtgcccatcattcccatcatttctccttggacattgatgttggatgtacagacttaaatgaggacttaggtgtatgggtgatattcaagattaagacgcaagatggccatgcaagactaggaaatctagaatttctcgaagagaaaccattagtaggagaagcactagctcgtgtgaaaagagcggagaaaaaatggagagacaaacgtgaaaaattggaatgggaaacaaatattgtttataaagaggcaaaagaatctgtagatgctttatttgtaaactctcaatatgatagattacaagcggataccaacatcgcgatgattcatgcggcagataaacgcgttcatagcattcgagaagcttatctgcctgagctgtctgtgattccgggtgtcaatgcggctatttttgaagaattagaagggcgtattttcactgcattctccctatatgatgcgagaaatgtcattaaaaatggtgattttaataatggcttatcctgctggaacgtgaaagggcatgtagatgtagaagaacaaaacaaccaccgttcggtccttgttgttccggaatgggaagcagaagtgtcacaagaagttcgtgtctgtccgggtcgtggctatatccttcgtgtcacagcgtacaaggagggatatggagaaggttgcgtaaccattcatgagatcgagaacaatacagacgaactgaagtttagcaactgtgtagaagaggaagtatatccaaacaacacggtaacgtgtaatgattatactgcgactcaagaagaatatgagggtacgtacacttctcgtaatcgaggatatgacggagcctatgaaagcaattcttctgtaccagctgattatgcatcagcctatgaagaaaaagcatatacagatggacgaagagacaatccttgtgaatctaacagaggatatggggattacacaccactaccagctggctatgtgacaaaagaattagagtacttcccagaaaccgataaggtatggattgagatcggagaaacggaaggaacattcatcgtggacagcgtggaattacttcttatggaggaataa

SEQ ID NO: 38 - protein, 1164 aa, synthetic construct
  REGION 1..1164: note = translated from synthesized coding region
MDNNPNINECIPYNCLSNPEEVLLDGERISTGNSSIDISLSLVQFLVSNFVPGGGFLVGLIDFVWGIVGPSQWDAFLVQIEQLINERIAEFARNAAIANLEGLGNNFNIYVEAFKEWEEDPKNPATRTRVIDRFRILDGLLERDIPSFRISGFEVPLLSVYAQAANLHLAILRDSVIFGERWGLTTINVNENYNRLIRHIDEYADHCANTYNRGLNNLPKSTYQDWITYNRLRRDLTLTVLDIAAFFPNYDNRRYPIQPVGQLTREVYTDPLINFNPQLQSVAQLPTFNVMENSAIRNPHLFDILNNLTIFTDWFSVGRNFYWGGHRVISSLIGGGNITSPIYGREANQEPPRSFTFNGPVFRTLSNPTLRLLQQPWPAPPFNLRGVEGVEFSTPTNSFTYRGRGTVDSLTELPPEDNSVPPREGYSHRLCHATFVQRSGTPFLTTGVVFSWTHRSATLTNTIDPERINQIPLVKGFRVWGGTSVITGPGFTGGDILRRNTFGDFVSLQVNINSPITQRYRLRFRYASSRDARVIVLTGAASTGVGGQVSVNMPLQKTMEIGENLTSRTFRYTDFSNPFSFRANPDIIGISEQPLFGAGSISSGELYIDKIEIILADATFEAESDLERAQKAVNALFTSSNQIGLKTDVTDYHIDRVSNLVECLSDEFCLDEKKELSEKVKHAKRLSDERNLLQDPNFRGINRQLDRGWRGSTDITIQGGDDVSKENYVTLLGTFDECYLTYLYQKIDESKLKAYTRYQLRGYIEDSQDLEIYLIRYNAKHETVNVPGTGSLWPLSAPSPIGKCAHHSHHFSLDIDVGCTDLNEDLGVWVIFKIKTQDGHARLGNLEFLEEKPLVGEALARVKRAEKKWRDKREKLEWETNIVYKEAKESVDALFVNSQYDRLQADTNIAMIHAADKRVHSIREAYLPELSVIPGVNAAIFEELEGRIFTAFSLYDARNVIKNGDFNNGLSCWNVKGHVDVEEQNNHRSVLVVPEWEAEVSQEVRVCPGRGYILRVTAYKEGYGEGCVTIHEIENNTDELKFSNCVEEEVYPNNTVTCNDYTATQEEYEGTYTSRNRGYDGAYESNSSVPADYASAYEEKAYTDGRRDNPCESNRGYGDYTPLPAGYVTKELEYFPETDKVWIEIGETEGTFIVDSVELLLMEE

SEQ ID NO: 39 - DNA, 2109 bp, synthetic construct
  misc_feature 1..2109: note = synthesized coding region
  source 1..2109: mol_type = other DNA
atggcacagagcagtaggatctgccacggtgtgcagaacccgtgcgtgatcatctcgaacctgagcaagtccaaccagaacaagtcaccgttctccgtgtccctcaagacccaccagcacccgagagcctacccgatcagcagctcctggggactgaagaagagtggcatgaccctgatcggctccgagctgagaccgctgaaggtgatgtccagcgtgtcagcggataacaacccgaacatcaacgagtgcatcccctacaactgcctgagcaaccccgaggaggtgctgctggacggcgagaggatctcaaccggcaacagcagcatcgacatcagcctgtccctggtgcagttcctggtgagcaacttcgtgccgggcggcggcttcctggtgggattaatcgacttcgtgtggggcatcgtcggcccgtcccagtgggacgccttcctggttcagatcgagcaattaattaatgaaaggatagcagagttcgcgaggaacgcggccatcgccaacctggagggcctgggcaacaacttcaacatctacgtggaagcatttaaggagtgggaggaggaccccaagaacccggccacgaggacgagggtgatcgaccgctttcgcatcctggacggcctgctggagagggacatcccgtccttcagaatcagcggcttcgaggtcccgctgctgtccgtgtacgcgcaagcggccaacctgcacctggcgatcctgagggactccgtgatattcggcgagaggtggggcctgaccaccatcaacgtgaatgaaaactacaaccggctgataaggcacatcgacgagtacgccgaccactgcgccaacacctacaataggggattaaataatctgcccaagagcacctaccaagactggatcacatataaccggctgaggagggacctgaccctgaccgtgctggacatcgccgcgttcttcccgaactacgacaataggcgctacccgatccagccggtgggccagctgacccgcgaggtgtacaccgacccattaattaatttcaacccgcagctccagtccgtggcccagctgccgaccttcaacgtgatggagaacagcgccatccggaacccgcacctgttcgacatcctgaataatctgaccatcttcaccgactggttctcagtgggccggaacttctactggggcggccatagggtgatctccagcctgatcggcggcggcaacatcacctccccgatctacgggagggaggcgaaccaggagccgccgaggtccttcaccttcaacggcccggtgtttaggaccctgtccaacccgaccctgaggctgctccagcagccgtggccggcgccgccgttcaacctgaggggcgtggagggcgtggagttcagcaccccgaccaacagcttcacctaccgggggaggggcaccgtggactcactgaccgagctgccgccggaggacaacagcgtgccgccgagggagggctacagccataggctgtgccacgccaccttcgtgcagaggagcggcaccccgttcttgacgaccggcgtggtgttctcctggacccaccggagcgcgaccctgaccaatacaatcgacccggagagaattaatcaaatcccgctggtgaagggcttccgggtgtggggcggcacctccgtgatcaccgggccgggctttaccggcggcgacatcctgaggaggaacacgttcggcgacttcgtgagcctccaagtgaacattaatagcccgatcacccagcgctaccggctgaggttccgctacgcgtcaagccgcgacgcgagggtgatcgtgctgaccggcgcggcctcaaccggcgtgggcggccaagtgtccgtgaacatgccgctgcaaaagacgatggagatcggcgagaacctgacctcaaggaccttccgctacaccgacttcagcaacccgttcagctttagggccaacccggatataatcggcatcagcgagcagccgctgttcggcgccggctccatctcaagcggcgagctgtacatcgataaaatcgagatcatcctggcggacgcgaccttggaggccgagtccgacctggagaggtga

SEQ ID NO: 40 - protein, 702 aa, synthetic construct
  REGION 1..702: note = translated from synthesized coding region
MAQSSRICHGVQNPCVIISNLSKSNQNKSPFSVSLKTHQHPRAYPISSSWGLKKSGMTLIGSELRPLKVMSSVSADNNPNINECIPYNCLSNPEEVLLDGERISTGNSSIDISLSLVQFLVSNFVPGGGFLVGLIDFVWGIVGPSQWDAFLVQIEQLINERIAEFARNAAIANLEGLGNNFNIYVEAFKEWEEDPKNPATRTRVIDRFRILDGLLERDIPSFRISGFEVPLLSVYAQAANLHLAILRDSVIFGERWGLTTINVNENYNRLIRHIDEYADHCANTYNRGLNNLPKSTYQDWITYNRLRRDLTLTVLDIAAFFPNYDNRRYPIQPVGQLTREVYTDPLINFNPQLQSVAQLPTFNVMENSAIRNPHLFDILNNLTIFTDWFSVGRNFYWGGHRVISSLIGGGNITSPIYGREANQEPPRSFTFNGPVFRTLSNPTLRLLQQPWPAPPFNLRGVEGVEFSTPTNSFTYRGRGTVDSLTELPPEDNSVPPREGYSHRLCHATFVQRSGTPFLTTGVVFSWTHRSATLTNTIDPERINQIPLVKGFRVWGGTSVITGPGFTGGDILRRNTFGDFVSLQVNINSPITQRYRLRFRYASSRDARVIVLTGAASTGVGGQVSVNMPLQKTMEIGENLTSRTFRYTDFSNPFSFRANPDIIGISEQPLFGAGSISSGELYIDKIEIILADATLEAESDLER